European Patent Specification EP 3 824 076 B1, published December 10, 2025. Title: IL-31 IMPROVES EFFICACY OF MACROPHAGE-BASED ADOPTIVE CELL THERAPY FOR CANCER. Applicant: ONCOHOST LTD LASTER, Morris C. The sequence listing filed with the application follows.

SEQUENCE LISTING (8 sequences)

SEQ ID NO: 1 - protein, 164 aa, Human
MASHSGPSTSVLFLFCCLGGWLASHTLPVRLLRPSDDVQKIVEELQSLSKMLLKDVEEEKGVLVSQNYTLPCLSPDAQPPNNIHSPAIRAYLKTIRQLDNKSVIDEIIEHLDKLIFQDAPETNISVPTDTHECKRFILTISQQFSECMDLALKSLTSGAQQATT

SEQ ID NO: 2 - DNA, 442 bp, Human
atggcctctcactcaggcccctcgacgtctgtgctctttctgttctgctgcctgggaggctggctggcctcccacacgttgcccgtccgtttactacgaccaagtggaaagatgtggaggaagagaagggcgtgctcgtgtcccagaattacacgctgccgtgtctcagccctgacgcccagccgccaaacaacatccacagcccagccatccgggcatatctcaagacaatcagacagctagacaacaaatctgttattgatgagatcatagagcacctcgacaaactcatatttcaagatgcaccagaaacaaacatttctgtgccaacagacacccatgaatgtaaacgcttcatcctgactatttctcaacagttttcagagtgcatggacctcgcactaaaatcattgacctctggagcccaacaggccaccactta

SEQ ID NO: 3 - DNA, 22 bp, Artificial Sequence
  ARG1 primer1
ctccaagccaaagtccttagag

SEQ ID NO: 4 - DNA, 22 bp, Artificial Sequence
  ARG1 primer2
aggagctgtcattagggacatc

SEQ ID NO: 5 - skipped
  iNOS primer1

SEQ ID NO: 6 - DNA, 19 bp, Artificial Sequence
  iNOS primer2
gtggacgggtcgatgtcac

SEQ ID NO: 7 - DNA, 22 bp, Artificial Sequence
  Hsp90 primer1
tcgtcagagctgatgatgaagt

SEQ ID NO: 8 - DNA, 23 bp, Artificial Sequence
  Hsp90 primer2
gcgtttaacccatccaactgaat